European Patent Application EP 4 523 702 A1, published March 19, 2025. Title: Combination of antibody-drug conjugate and anti-SIRP alpha antibody. Applicant: DAIICHI SANKYO COMPANY, LTD. Application JP. The sequence listing filed with the application follows.

SEQUENCE LISTING (13 sequences)

SEQ ID NO: 1 - protein, 466 aa, synthetic construct
  REGION 1..466: note = Amino acid sequence of hH1 heavy chain of humanized anti-SIRP alpha antibody hD13
MKHLWFFLLLVAAPRWVLSQVQLVESGGGVVQPGRSLRLSCAASGFTFSDYGMIWVRQAPGKGLEWVASISSSSSYIYYADSVKGRFTISRDNSKNRLYLQMNSLRAEDTAVYYCARRYYGFNYPFDYWGQGTMVTVSSASTKGPSVFPLAPCSRSTSESTAALGCLVKDYFPEPVTVSWNSGALTSGVHTFPAVLQSSGLYSLSSVVTVPSSSLGTKTYTCNVDHKPSNTKVDKRVESKYGPPCPPCPAPEAAGGPSVFLFPPKPKDTLMISRTPEVTCVVVDVSQEDPEVQFNWYVDGVEVHNAKTKPREEQFNSTYRVVSVLTVLHQDWLNGKEYKCKVSNKGLPSSIEKTISKAKGQPREPQVYTLPPSQEEMTKNQVSLTCLVKGFYPSDIAVEWESNGQPENNYKTTPPVLDSDGSFFLYSRLTVDKSRWQEGNVFSCSVMHEALHNHYTQKSLSLSLGK

SEQ ID NO: 2 - protein, 466 aa, synthetic construct
  REGION 1..466: note = Amino acid sequence of hH2 heavy chain of humanized anti-SIRP alpha antibody hD13
MKHLWFFLLLVAAPRWVLSEVQLVESGGGVVQPGRSLRLSCAASGFTFSDYGMIWVRQAPGKGLEWVASISSSSSYIYYADSVKGRFTISRDNSKNTLYLQMNSLRAEDTAVYYCARRYYGFNYPFDYWGQGTMVTVSSASTKGPSVFPLAPCSRSTSESTAALGCLVKDYFPEPVTVSWNSGALTSGVHTFPAVLQSSGLYSLSSVVTVPSSSLGTKTYTCNVDHKPSNTKVDKRVESKYGPPCPPCPAPEAAGGPSVFLFPPKPKDTLMISRTPEVTCVVVDVSQEDPEVQFNWYVDGVEVHNAKTKPREEQFNSTYRVVSVLTVLHQDWLNGKEYKCKVSNKGLPSSIEKTISKAKGQPREPQVYTLPPSQEEMTKNQVSLTCLVKGFYPSDIAVEWESNGQPENNYKTTPPVLDSDGSFFLYSRLTVDKSRWQEGNVFSCSVMHEALHNHYTQKSLSLSLGK

SEQ ID NO: 3 - protein, 234 aa, synthetic construct
  REGION 1..234: note = Amino acid sequence of hL2 light chain of humanized anti-SIRP alpha antibody hD13
MVLQTQVFISLLLWISGAYGAIQLTQSPSSLSASVGQRVTITCGASKSVRTYMHWYQQKPGKAPKLLIYSASNLEAGVPSRFSGSGSGTDFTLTISSLQPEDFATYYCQQSNEPPYTFGQGTKLEIKRTVAAPSVFIFPPSDEQLKSGTASVVCLLNNFYPREAKVQWKVDNALQSGNSQESVTEQDSKDSTYSLSSTLTLSKADYEKHKVYACEVTHQGLSSPVTKSFNRGEC

SEQ ID NO: 4 - protein, 234 aa, synthetic construct
  REGION 1..234: note = Amino acid sequence of hL3 light chain of humanized anti-SIRP alpha antibody hD13
MVLQTQVFISLLLWISGAYGDTQLTQSPSSLSASVGQRVTITCGASKSVRTYMHWYQQKPGKQPKLLIYSASNLEAGVPSRFSGSGSGTDFTLTISSLQPEDFATYYCQQSNEPPYTFGQGTKLEIKRTVAAPSVFIFPPSDEQLKSGTASVVCLLNNFYPREAKVQWKVDNALQSGNSQESVTEQDSKDSTYSLSSTLTLSKADYEKHKVYACEVTHQGLSSPVTKSFNRGEC

SEQ ID NO: 5 - protein, 234 aa, synthetic construct
  REGION 1..234: note = Amino acid sequence of hL4 light chain of humanized anti-SIRP alpha antibody hD13
MVLQTQVFISLLLWISGAYGDTVLTQSPDSLAVSLGQRATINCGASKSVRTYMHWYQQKPGQQPKLLIYSASNLEAGVPSRFSGSGSGTDFTLTISSLQAEDVAVYYCQQSNEPPYTFGQGTKVEIKRTVAAPSVFIFPPSDEQLKSGTASVVCLLNNFYPREAKVQWKVDNALQSGNSQESVTEQDSKDSTYSLSSTLTLSKADYEKHKVYACEVTHQGLSSPVTKSFNRGEC

SEQ ID NO: 6 - protein, 10 aa, synthetic construct
  REGION 1..10: note = Amino acid sequence of CDR-H1 of chimeric anti-SIRP alpha antibody cD13
GFTFSDYGMI

SEQ ID NO: 7 - protein, 10 aa, synthetic construct
  REGION 1..10: note = Amino acid sequence of CDR-H2 of chimeric anti-SIRP alpha antibody cD13
SISSSSSYIY

SEQ ID NO: 8 - protein, 11 aa, synthetic construct
  REGION 1..11: note = Amino acid sequence of CDR-H3 of chimeric anti-SIRP alpha antibody cD13
RYYGFNYPFDY

SEQ ID NO: 9 - protein, 11 aa, synthetic construct
  REGION 1..11: note = Amino acid sequence of CDR-L1 of chimeric anti-SIRP alpha antibody cD13
GASKSVRTYMH

SEQ ID NO: 10 - protein, 7 aa, synthetic construct
  REGION 1..7: note = Amino acid sequence of CDR-L2 of chimeric anti-SIRP alpha antibody cD13
SASNLEA

SEQ ID NO: 11 - protein, 9 aa, synthetic construct
  REGION 1..9: note = Amino acid sequence of CDR-L3 of chimeric anti-SIRP alpha antibody cD13
QQSNEPPYT

SEQ ID NO: 12 - protein, 460 aa, Mus musculus
MKHLWFFLLLVAAPRWVLSEVQLVESGGGLVQPGGSLKLSCAASGFTFSNYDMAWVRQAPTKGLEWVASISTRGGSSYYRDSVKGRFTVSRDNAKSTLYLQMDSLRSEDTATYYCARHPGDYFDYWGQGVMVTVSSAKTTPPSVYPLAPGSAAQTNSMVTLGCLVKGYFPEPVTVTWNSGSLSSGVHTFPAVLQSDLYTLSSSVTVPSSTWPSETVTCNVAHPASSTKVDKKIVPRDCGCKPCICTVPEVSSVFIFPPKPKDVLTITLTPKVTCVVVAISKDDPEVQFSWFVDDVEVHTAQTQPREEQFNSTFRSVSELPIMHQDWLNGKEFKCRVNSAAFPAPIEKTISKTKGRPKAPQVYTIPPPKEQMAKDKVSLTCMITDFFPEDITVEWQWNGQPAENYKNTQPIMDTDGSYFVYSKLNVQKSNWEAGNTFTCSVLHEGLHNHHTEKSLSHSPGK

SEQ ID NO: 13 - protein, 233 aa, Mus musculus
MVLQTQVFISLLLWISGAYGDTVLTQSPALAVSPGERVTISCRASESVSTLIHWYQQKPGQQPKLLIYLTSHLESGVPARFSGSGSGTDFTLTIDPVEADDTATYYCQQSWTHPWTFGGGTKLELKRADAAPTVSIFPPSSEQLTSGGASVVCFLNNFYPKDINVKWKIDGSERQNGVLNSWTDQDSKDSTYSMSSTLTLTKDEYERHNSYTCEATHKTSTSPIVKSFNRNEC